European Patent Application EP 4 574 978 A1, published June 25, 2025. Title: DNA aptamer having affinity for PD-1 protein and its use. Applicant: Uniwersytet Jagiellonski. The sequence listing filed with the application follows.

SEQUENCE LISTING (6 sequences)

SEQ ID NO: 1 - DNA, 88 bp, synthetic construct
  source 1..88: mol_type = other DNA
catgcttccccagggagatgcggggggtgggagggtggagcagctgtggttggtgtggttggaccctggaggaacatgcgtcgcaaac

SEQ ID NO: 2 - DNA, 68 bp, synthetic construct
  source 1..68: mol_type = other DNA
catgcttccccagggagatgcggggggtgggagggtggagcagctgtggttggtgtggttggaccctg

SEQ ID NO: 3 - DNA, 90 bp, synthetic construct
  source 1..90: mol_type = other DNA
catgcttccccagggagatgnnnnnnnnnnnnnnnnnnnnnnnnnnnnnnnnnnnnnnnnnnnnnnnnnngaggaacatgcgtcgcaaac

SEQ ID NO: 4 - DNA, 20 bp, synthetic construct
  source 1..20: mol_type = other DNA
catgcttccccagggagatg

SEQ ID NO: 5 - DNA, 20 bp, synthetic construct
  source 1..20: mol_type = other DNA
gtttgcgacgcatgttcctc

SEQ ID NO: 6 - DNA, 16 bp, synthetic construct
  source 1..16: mol_type = other DNA
aaaaccccttttgggg